European Patent Application EP 4 302 777 A1, published January 10, 2024. Title: ANTI-CLDN6 ANTIBODY AND USE THEREOF. Applicant: SHANGHAI GENBASE BIOTECHNOLOGY CO., LTD. The sequence listing filed with the application follows.

SEQUENCE LISTING (33 sequences)

SEQ ID NO: 1 - protein, 116 aa, artificial
  15H2 heavy chain variable region
DVQLQESGPGLVKPSQSLSLTCSVTGYSITSGYYWNWIRQFPGNKLEWMGYISYDGSNNYNPSLKNRFSIIRDTSKNQFFLKFNSVTTEDTATYYCARGGYYFDYWGQGTTLTVSS

SEQ ID NO: 2 - protein, 113 aa, artificial
  15H2 light chain variable region
DIVMTQSPSSLAMSVGQKVTMSCKSSQSLLNTNNQKNYLAWYQQKPGQSPKLLVYFASTRESGVPDRFIGSGSGTDFTLTISSVQAEDLADYFCQQHYNAPRTFGGGTKLEIK

SEQ ID NO: 3 - protein, 9 aa, artificial
  15H2 HCDR1
GYSITSGYY

SEQ ID NO: 4 - protein, 7 aa, artificial
  15H2 HCDR2
ISYDGSN

SEQ ID NO: 5 - protein, 9 aa, artificial
  15H2 HCDR3
ARGGYYFDY

SEQ ID NO: 6 - protein, 12 aa, artificial
  15H2 LCDR1
QSLLNTNNQKNY

SEQ ID NO: 7 - protein, 7 aa, artificial
  15H2 LCDR2
FASTRES

SEQ ID NO: 8 - protein, 9 aa, artificial
  15H2 LCDR3
QQHYNAPRT

SEQ ID NO: 9 - protein, 121 aa, artificial
  7008-03 heavy chain variable region
EVQLVESGGGLVQPGGSLRLSCAASGFTFSIYGMSWVRQAPGKGLEWVATISRDASYTYFPDSVKGRFTISRDNAKNSLYLQMNSLRAEDTAVYYCVRLGDNDRGYAMDYWGQGTLVTVSS

SEQ ID NO: 10 - protein, 112 aa, artificial
  7008-03 light chain variable region
DVVMTQSPLSLPVTLGQPASISCRSSQSVVHVNANTYLEWYQQRPGQSPRLLIYKVSNRFPGVPDRFSGSGSGTDFTLKISRVEAEDVGVYYCFQGSHVPRTFGGGTKVEIK

SEQ ID NO: 11 - protein, 121 aa, artificial
  9H3 heavy chain variable region
EVQLVESGGDLVKPGGSLKLSCAASGFTFSIYGMSWVRQSPDRRLEWVATISRDGSYTYFPDSVKGRFTISRDNAKNTLYLQMSSLKSEDTAMYYCVRLGDNDRGYAMDYWGQGTSVTVSS

SEQ ID NO: 12 - protein, 112 aa, artificial
  9H3 light chain variable region
DVLMTQTPLSLPVSLGDQASISCRSSQSVVHVNGNTYLEWYLQKPGQSPRLLIYKVSNRFPGVPDRFSGSGSGTDFTLRISRVEAEDLGVYYCFQGSHVPRTFGGGTNLEIK

SEQ ID NO: 13 - protein, 8 aa, artificial
  9H3 HCDR1
GFTFSIYG

SEQ ID NO: 14 - protein, 8 aa, artificial
  9H3 HCDR2
ISRDGSYT

SEQ ID NO: 15 - protein, 14 aa, artificial
  9H3 HCDR3
VRLGDNDRGYAMDY

SEQ ID NO: 16 - protein, 11 aa, artificial
  9H3 LCDR1
QSVVHVNGNTY

SEQ ID NO: 17 - protein, 7 aa, artificial
  9H3 LCDR2
KVSNRFP

SEQ ID NO: 18 - protein, 9 aa, artificial
  9H3 LCDR3
FQGSHVPRT

SEQ ID NO: 19 - protein, 116 aa, artificial
  7008-01 heavy chain variable region
QVQLQESGPGLVKPSETLSLTCTVSGYSITSGYYWNWIRQPPGKGLEWMGYISYSGSNNYNPSLKNRVTISRDTSKNQFSLKLSSVTAADTAVYYCARGGYYFDYWGQGTLVTVSS

SEQ ID NO: 20 - protein, 113 aa, artificial
  7008-01 light chain variable region
DIVMTQSPDSLAVSLGERATINCKSSQSLLNTNNQKNYLAWYQQKPGQPPKLLIYFASTRESGVPDRFSGSGSGTDFTLTISSLQAEDVAVYFCQQHYNAPRTFGGGTKVEIK

SEQ ID NO: 21 - protein, 330 aa, artificial
  Human IgG1 heavy chain constant region
ASTKGPSVFPLAPSSKSTSGGTAALGCLVKDYFPEPVTVSWNSGALTSGVHTFPAVLQSSGLYSLSSVVTVPSSSLGTQTYICNVNHKPSNTKVDKKVEPKSCDKTHTCPPCPAPELLGGPSVFLFPPKPKDTLMISRTPEVTCVVVDVSHEDPEVKFNWYVDGVEVHNAKTKPREEQYNSTYRVVSVLTVLHQDWLNGKEYKCKVSNKALPAPIEKTISKAKGQPREPQVYTLPPSREEMTKNQVSLTCLVKGFYPSDIAVEWESNGQPENNYKTTPPVLDSDGSFFLYSKLTVDKSRWQQGNVFSCSVMHEALHNHYTQKSLSLSPGK

SEQ ID NO: 22 - protein, 107 aa, artificial [sequence omitted]

SEQ ID NO: 23 - protein, 8 aa, artificial
  7008-03 HCDR2
ISRDASYT

SEQ ID NO: 24 - protein, 11 aa, artificial
  7008-03 LCDR1
QSVVHVNANTY

SEQ ID NO: 25 - DNA, 348 bp, artificial
  Nucleic acid sequence encoding 15H2 heavy chain variable region
gatgtacagcttcaggagtcaggacctggcctcgtgaaaccttctcagtctctgtctctcacctgctctgtcactggctactccatcaccagtggttattactggaactggatccggcagtttccaggaaacaaactggaatggatgggctacataagctacgacggtagcaataactacaacccatctctcaaaaatcgattctccatcattcgtgacacatctaagaaccagtttttcctgaagttcaattctgtgactactgaggacacagctacatattactgcgccaggggggggtactactttgactactggggccaaggcaccactctcacagtctcctca

SEQ ID NO: 26 - DNA, 339 bp, artificial
  Nucleic acid sequence encoding 15H2 light chain variable region
gacattgtgatgacacagtctccatcctccctggctatgtcagtaggacagaaggtcactatgagctgcaagtccagtcagagccttttaaatactaacaatcaaaagaactatttggcctggtaccagcagaaaccaggacagtctcctaaacttctggtatactttgcatccactagggagtctggggtccctgatcgcttcataggcagtggatctgggacagatttcactcttaccatcagcagtgtgcaggctgaagacctggcagattacttctgtcaacaacattataacgctcctcggacgttcggtggaggcaccaagctggaaatcaaa

SEQ ID NO: 27 - DNA, 363 bp, artificial
  Nucleic acid sequence encoding 9H3 heavy chain variable region
gaggtgcagctggtggaatctgggggagacttagtgaagcctggagggtccctgaaactctcctgtgcagcctctggattcactttcagtatctatggcatgtcttgggttcgccagagtccagacaggaggctggaatgggtcgcaaccattagtcgtgatggtagttacacctactttccagacagtgtgaaggggcgattcaccatctccagagacaatgccaagaacaccctgtatttgcaaatgagcagtctgaagtctgaggacacagccatgtattactgtgtaagactgggtgataacgacaggggctatgctatggactactggggtcaaggaacttcagtcaccgtctcctca

SEQ ID NO: 28 - DNA, 336 bp, artificial
  Nucleic acid sequence encoding 9H3 light chain variable region
gatgttttgatgacccaaactccactctccctgcctgtcagtcttggagatcaagcctccatctcttgcagatctagtcagagtgttgtacatgttaatggaaacacctatttagaatggtacctgcagaaaccaggccagtctccaaggctcctgatctacaaagtttccaaccgctttcctggggtcccagacaggttcagtggcagtggatcagggacagatttcacactcaggatcagcagagtggaggctgaggatctgggagtttattactgctttcaaggttcacatgttcctcggacgttcggtggaggcaccaacctggaaatcaaa

SEQ ID NO: 29 - DNA, 348 bp, artificial
  Nucleic acid sequence encoding 7008-01 heavy chain variable region
caggtgcagctgcaggagagcggccccggactggtgaagccctcagagacactgagcctgacatgcacagtgagcggctactccattacaagcggctactactggaactggatcagacagccccccggcaagggcctggaatggatgggctatatctcctacagcggcagcaacaactacaaccccagcctgaagaacagggtgaccatctctcgcgacacctccaagaaccagttctccctgaagctgagtagcgtgactgccgctgacaccgccgtgtactattgcgccagaggcggctactacttcgactactggggccagggcaccctggtgaccgtgagcagc

SEQ ID NO: 30 - DNA, 339 bp, artificial
  Nucleic acid sequence encoding 7008-01 light chain variable region
gacattgtgatgacccagagccccgactccctggccgtgagcctgggagaaagagccaccatcaactgcaagagcagccagagcctgctgaacaccaacaaccagaaaaactacctggcctggtaccagcagaaacccggccagccccccaaactgctgatctacttcgcctccacccgcgagtccggcgtgcctgatagattctccggcagcggcagcggcaccgacttcaccctgactatcagcagcctgcaggctgaggacgtggccgtgtacttctgccagcagcattacaacgctcccagaacctttggaggaggcaccaaggtggaaatcaag

SEQ ID NO: 31 - DNA, 363 bp, artificial
  Nucleic acid sequence encoding 7008-03 heavy chain variable region
gaggtgcagctggtggagagcggggggggactggtgcagccaggaggaagcctgagactgagctgtgccgccagcgggtttacatttagcatttatgggatgtcctgggtgagacaggcccccggaaaaggactggagtgggtggctactatcagcagagacgctagctacacctacttccccgattccgtgaagggcagattcacaatcagcagagataacgctaagaacagcctgtatctgcagatgaacagcctgcgggccgaggacacagccgtgtattactgcgtgaggctgggcgacaacgatagaggatacgccatggactactgggggcagggaacactggtgaccgtgagcagc

SEQ ID NO: 32 - DNA, 336 bp, artificial
  Nucleic acid sequence encoding 7008-03 light chain variable region
gacgtggtgatgacccagagccccctgagcctgcccgtgaccctgggacagcccgctagtatcagctgcagaagcagccagagcgtggtgcacgtgaacgccaacacatatctggagtggtatcagcagaggcctggacagagccccagactgctgatctacaaggtgagcaacagattcccaggcgtgccagacagattctctggaagcggcagcggaacagactttaccctgaagatctccagagtggaggccgaggacgtgggagtgtactactgcttccagggcagccacgtgcccagaacattcggcggcggcaccaaagtggagatcaaa

SEQ ID NO: 33 - protein, 7 aa, artificial
  7008-01 HCDR2
ISYSGSN